European Patent Application EP 4 588 933 A2, published July 23, 2025. Title: Wasch- und Reinigungsmittel mit verbesserter Enzym-Stabilität. Applicant: Henkel AG & Co. KGaA. The sequence listing filed with the application follows.

SEQUENCE LISTING (25 sequences)

SEQ ID NO: 1 - protein, 269 aa, Bacillus gibsonii
QQTVPWGITRVQAPTVHNRGITGSGVKVAILDTGIAQHSDLTIRGGASFVPGESTTADLNGHGTHVAGTVAALNNSIGVIGVAPSADLYAVKVLGANGRGSVSGIAQGLEWAATNNMHIANMSLGSDAPSTTLERAVNYATSRGVLVIAATGNNGTGSIGYPARYANAMAVGATDQNNRRASFSQYGTGIDIVAPGVGIQSTYLNNSYASMPGTSMATPHVAGVAALVKQKNPSWNATQIRNHLKNTATNLGNSSQFGSGLVNADAATR

SEQ ID NO: 2 - protein, 4 aa, synthetic construct
  REGION 1..4: note = enzyme stabilizer
  MOD_RES 1: note = Ac-Leu
  MOD_RES 4: note = Tyr-H
LGAY

SEQ ID NO: 3 - protein, 4 aa, synthetic construct
  REGION 1..4: note = enzyme stabilizer
  MOD_RES 1: note = Ac-Phe
  MOD_RES 4: note = Leu-H
FGAL

SEQ ID NO: 4 - protein, 4 aa, synthetic construct
  REGION 1..4: note = enzyme stabilizer
  MOD_RES 1: note = Ac-Phe
  MOD_RES 4: note = Phe-H
FGAF

SEQ ID NO: 5 - protein, 4 aa, synthetic construct
  REGION 1..4: note = enzyme stabilizer
  MOD_RES 1: note = Ac-Phe
  MOD_RES 4: note = Tyr-H
FGVY

SEQ ID NO: 6 - protein, 4 aa, synthetic construct
  REGION 1..4: note = enzyme stabilizer
  MOD_RES 1: note = Ac-Phe
  MOD_RES 4: note = Met-H
FGAM

SEQ ID NO: 7 - protein, 4 aa, synthetic construct
  REGION 1..4: note = enzyme stabilizer
  MOD_RES 1: note = Ac-Trp
  MOD_RES 4: note = Tyr-H
WLVY

SEQ ID NO: 8 - protein, 4 aa, synthetic construct
  REGION 1..4: note = enzyme stabilizer
  MOD_RES 1: note = MeO-CO-Phe
  MOD_RES 4: note = Leu-H
FGAL

SEQ ID NO: 9 - protein, 4 aa, synthetic construct
  REGION 1..4: note = enzyme stabilizer
  MOD_RES 1: note = MeO-CO-Phe
  MOD_RES 4: note = Phe-H
FGAF

SEQ ID NO: 10 - protein, 5 aa, synthetic construct
  REGION 1..5: note = enzyme stabilizer
  SITE 2: note = MISC_FEATURE - urea
  MOD_RES 5: note = Tyr-H
FXRVY

SEQ ID NO: 11 - protein, 5 aa, synthetic construct
  REGION 1..5: note = enzyme stabilizer
  SITE 2: note = MISC_FEATURE - urea
  MOD_RES 5: note = Tyr-H
FXGGY

SEQ ID NO: 12 - protein, 5 aa, synthetic construct
  REGION 1..5: note = enzyme stabilizer
  SITE 2: note = MISC_FEATURE - urea
  MOD_RES 5: note = Phe-H
FXGAF

SEQ ID NO: 13 - protein, 5 aa, synthetic construct
  REGION 1..5: note = enzyme stabilizer
  SITE 2: note = MISC_FEATURE - urea
  MOD_RES 5: note = Tyr-H
FXGAY

SEQ ID NO: 14 - protein, 5 aa, synthetic construct
  REGION 1..5: note = enzyme stabilizer
  SITE 2: note = MISC_FEATURE - urea
  MOD_RES 5: note = Leu-H
FXGAL

SEQ ID NO: 15 - skipped

SEQ ID NO: 16 - protein, 5 aa, synthetic construct
  REGION 1..5: note = enzyme stabilizer
  SITE 2: note = MISC_FEATURE - urea
  MOD_RES 5: note = Tyr-H
YXRVY

SEQ ID NO: 17 - protein, 5 aa, synthetic construct
  REGION 1..5: note = enzyme stabilizer
  SITE 2: note = MISC_FEATURE - urea
  MOD_RES 5: note = Tyr-H
YXGAY

SEQ ID NO: 18 - protein, 6 aa, synthetic construct
  REGION 1..6: note = enzyme stabilizer
  MOD_RES 6: note = Phe-H
FCSRVF

SEQ ID NO: 19 - protein, 6 aa, synthetic construct
  REGION 1..6: note = enzyme stabilizer
  MOD_RES 6: note = Tyr-H
FCSRVY

SEQ ID NO: 20 - protein, 6 aa, synthetic construct
  REGION 1..6: note = enzyme stabilizer
  MOD_RES 6: note = Tyr-H
FCSGAY

SEQ ID NO: 21 - protein, 4 aa, synthetic construct
  REGION 1..4: note = enzyme stabilizer
  MOD_RES 1: note = Ac-Phe
  MOD_RES 4: note = Tyr-H
FGAY

SEQ ID NO: 22 - protein, 4 aa, synthetic construct
  REGION 1..4: note = enzyme stabilizer
  MOD_RES 1: note = Ac-Tyr
  MOD_RES 4: note = Tyr-H
YGAY

SEQ ID NO: 23 - protein, 4 aa, synthetic construct
  REGION 1..4: note = enzyme stabilizer
  MOD_RES 1: note = MeSO2-Phe
  MOD_RES 4: note = Leu-H
FGAL

SEQ ID NO: 24 - protein, 4 aa, synthetic construct
  REGION 1..4: note = enzyme stabilizer
  MOD_RES 1: note = EtSO2-Phe
  MOD_RES 4: note = Leu-H
FGAL

SEQ ID NO: 25 - protein, 4 aa, synthetic construct
  REGION 1..4: note = enzyme stabilizer
  MOD_RES 1: note = MeO(OH)(O)P-Leu
  MOD_RES 4: note = Leu-H
LGAL